European Patent Specification EP 4 326 312 B1, published September 16, 2026. Title: Method of treating lower urinary tract symptoms. Applicant: Versameb AG. The sequence listing filed with the application follows.

SEQUENCE LISTING (16 sequences)

SEQ ID NO: 1 - DNA, 81 bp, Artificial Sequence
  pro-domain of human IGF1
gtgaagatgcacaccatgagcagcagccacctgttctatctggccctgtgcctgctgacctttaccagctctgctaccgcc

SEQ ID NO: 2 - DNA, 210 bp, Artificial Sequence
  mature human IGF1
ggacctgagacactttgtggcgctgaactggtggacgccctgcagtttgtgtgtggcgacagaggcttctacttcaacaagcccacaggctacggcagcagctctagaagggctcctcagaccggaatcgtggacgagtgctgcttcagaagctgcgacctgcggcggctggaaatgtattgtgcccctctgaagcctgccaagagcgcc

SEQ ID NO: 3 - protein, 18 aa, Homo sapiens
MTILFLTMVISYFGCMKA

SEQ ID NO: 4 - DNA, 54 bp, Artificial Sequence
  signal peptide of human BDNF
atgaccatcctgtttctgacaatggtcatcagctacttcggctgcatgaaggcc

SEQ ID NO: 5 - DNA, 63 bp, Artificial Sequence
  signal peptide of human Insulin growth factor 1 (IGF1)
atgggcaagattagcagcctgcctacacagctgttcaagtgctgcttctgcgacttcctgaaa

SEQ ID NO: 6 - protein, 21 aa, Homo sapiens
MGKISSLPTQLFKCCFCDFLK

SEQ ID NO: 7 - DNA, 348 bp, Artificial Sequence
  DNA sequence of Cpd.1A and Cpd.1B
atgaccatcctgtttctgacaatggtcatcagctacttcggctgcatgaaggccgtgaagatgcacaccatgagcagcagccacctgttctatctggccctgtgcctgctgacctttaccagctctgctaccgccggacctgagacactttgtggcgctgaactggtggacgccctgcagtttgtgtgtggcgacagaggcttctacttcaacaagcccacaggctacggcagcagctctagaagggctcctcagaccggaatcgtggacgagtgctgcttcagaagctgcgacctgcggcggctggaaatgtattgtgcccctctgaagcctgccaagagcgcctaa

SEQ ID NO: 8 - RNA, 348 nt, Artificial Sequence
  RNA sequence of Cpd.1A and Cpd.1B
  misc_feature (1)..(348): m1f (uridine is 1-methylpseudouridine)
augaccauccuguuucugacaauggucaucagcuacuucggcugcaugaaggccgugaagaugcacaccaugagcagcagccaccuguucuaucuggcccugugccugcugaccuuuaccagcucugcuaccgccggaccugagacacuuuguggcgcugaacugguggacgcccugcaguuuguguguggcgacagaggcuucuacuucaacaagcccacaggcuacggcagcagcucuagaagggcuccucagaccggaaucguggacgagugcugcuucagaagcugcgaccugcggcggcuggaaauguauugugccccucugaagccugccaagagcgccuaa

SEQ ID NO: 9 - DNA, 2740 bp, Artificial Sequence
  DNA sequence of vector pMA-T with Cpd.1A
ctaaattgtaagcgttaatattttgttaaaattcgcgttaaatttttgttaaatcagctcattttttaaccaataggccgaaatcggcaaaatcccttataaatcaaaagaatagaccgagatagggttgagtggccgctacagggcgctcccattcgccattcaggctgcgcaactgttgggaagggcgtttcggtgcgggcctcttcgctattacgccagctggcgaaagggggatgtgctgcaaggcgattaagttgggtaacgccagggttttcccagtcacgacgttgtaaaacgacggccagtgagcgcgacgtaatacgactcactatagggcgaattggcggaaggccgtcaaggccacgtgtcttgtccagagctcggatccgccaccatgaccatcctgtttctgacaatggtcatcagctacttcggctgcatgaaggccgtgaagatgcacaccatgagcagcagccacctgttctatctggccctgtgcctgctgacctttaccagctctgctaccgccggacctgagacactttgtggcgctgaactggtggacgccctgcagtttgtgtgtggcgacagaggcttctacttcaacaagcccacaggctacggcagcagctctagaagggctcctcagaccggaatcgtggacgagtgctgcttcagaagctgcgacctgcggcggctggaaatgtattgtgcccctctgaagcctgccaagagcgcctaagaattcggtacctggagcacaagactggcctcatgggccttccgctcactgcccgctttccagtcgggaaacctgtcgtgccagctgcattaacatggtcatagctgtttccttgcgtattgggcgctctccgcttcctcgctcactgactcgctgcgctcggtcgttcgggtaaagcctggggtgcctaatgagcaaaaggccagcaaaaggccaggaaccgtaaaaaggccgcgttgctggcgtttttccataggctccgcccccctgacgagcatcacaaaaatcgacgctcaagtcagaggtggcgaaacccgacaggactataaagataccaggcgtttccccctggaagctccctcgtgcgctctcctgttccgaccctgccgcttaccggatacctgtccgcctttctcccttcgggaagcgtggcgctttctcatagctcacgctgtaggtatctcagttcggtgtaggtcgttcgctccaagctgggctgtgtgcacgaaccccccgttcagcccgaccgctgcgccttatccggtaactatcgtcttgagtccaacccggtaagacacgacttatcgccactggcagcagccactggtaacaggattagcagagcgaggtatgtaggcggtgctacagagttcttgaagtggtggcctaactacggctacactagaagaacagtatttggtatctgcgctctgctgaagccagttaccttcggaaaaagagttggtagctcttgatccggcaaacaaaccaccgctggtagcggtggtttttttgtttgcaagcagcagattacgcgcagaaaaaaaggatctcaagaagatcctttgatcttttctacggggtctgacgctcagtggaacgaaaactcacgttaagggattttggtcatgagattatcaaaaaggatcttcacctagatccttttaaattaaaaatgaagttttaaatcaatctaaagtatatatgagtaaacttggtctgacagttaccaatgcttaatcagtgaggcacctatctcagcgatctgtctatttcgttcatccatagttgcctgactccccgtcgtgtagataactacgatacgggagggcttaccatctggccccagtgctgcaatgataccgcgagaaccacgctcaccggctccagatttatcagcaataaaccagccagccggaagggccgagcgcagaagtggtcctgcaactttatccgcctccatccagtctattaattgttgccgggaagctagagtaagtagttcgccagttaatagtttgcgcaacgttgttgccattgctacaggcatcgtggtgtcacgctcgtcgtttggtatggcttcattcagctccggttcccaacgatcaaggcgagttacatgatcccccatgttgtgcaaaaaagcggttagctccttcggtcctccgatcgttgtcagaagtaagttggccgcagtgttatcactcatggttatggcagcactgcataattctcttactgtcatgccatccgtaagatgcttttctgtgactggtgagtactcaaccaagtcattctgagaatagtgtatgcggcgaccgagttgctcttgcccggcgtcaatacgggataataccgcgccacatagcagaactttaaaagtgctcatcattggaaaacgttcttcggggcgaaaactctcaaggatcttaccgctgttgagatccagttcgatgtaacccactcgtgcacccaactgatcttcagcatcttttactttcaccagcgtttctgggtgagcaaaaacaggaaggcaaaatgccgcaaaaaagggaataagggcgacacggaaatgttgaatactcatactcttcctttttcaatattattgaagcatttatcagggttattgtctcatgagcggatacatatttgaatgtatttagaaaaataaacaaataggggttccgcgcacatttccccgaaaagtgccac

SEQ ID NO: 10 - DNA, 2894 bp, Artificial Sequence
  DNA sequence of vector pMK with Cpd.1B
ctaaattgtaagcgttaatattttgttaaaattcgcgttaaatttttgttaaatcagctcattttttaaccaataggccgaaatcggcaaaatcccttataaatcaaaagaatagaccgagatagggttgagtggccgctacagggcgctcccattcgccattcaggctgcgcaactgttgggaagggcgtttcggtgcgggcctcttcgctattacgccagctggcgaaagggggatgtgctgcaaggcgattaagttgggtaacgccagggttttcccagtcacgacgttgtaaaacgacggccagtgagcgcgacgtaatacgactcactatagggcgaattgaaggaaggccgtcaaggccgcatgtcttgtccagagctcggatccgccaccatgaccatcctgtttctgacaatggtcatcagctacttcggctgcatgaaggccgtgaagatgcacaccatgagcagcagccacctgttctatctggccctgtgcctgctgacctttaccagctctgctaccgccggacctgagacactttgtggcgctgaactggtggacgccctgcagtttgtgtgtggcgacagaggcttctacttcaacaagcccacaggctacggcagcagctctagaagggctcctcagaccggaatcgtggacgagtgctgcttcagaagctgcgacctgcggcggctggaaatgtattgtgcccctctgaagcctgccaagagcgcctaagaattcggtacctggagcacaagactggcctcatgggccttccgctcactgcccgctttccagtcgggaaacctgtcgtgccagctgcattaacatggtcatagctgaaaaaaaaaaaaaaaaaaaaaaaaaaaaaaaaaaaaaaaaaaaaaaaaaaaaaaaaaaaaaaaaaaaaaaaaaaaaaaaaaaaaaaaaaaaaaaaaaaaaaaaaaaaaaaaaaaaaaaaactcgaggctcttcctgggcctcatgggccttcctttcactgcccgctttccagtcgggaaacctgtcgtgccagctgcattaacatggtcatagctgtttccttgcgtattgggcgctctccgcttcctcgctcactgactcgctgcgctcggtcgttcgggtaaagcctggggtgcctaatgagcaaaaggccagcaaaaggccaggaaccgtaaaaaggccgcgttgctggcgtttttccataggctccgcccccctgacgagcatcacaaaaatcgacgctcaagtcagaggtggcgaaacccgacaggactataaagataccaggcgtttccccctggaagctccctcgtgcgctctcctgttccgaccctgccgcttaccggatacctgtccgcctttctcccttcgggaagcgtggcgctttctcatagctcacgctgtaggtatctcagttcggtgtaggtcgttcgctccaagctgggctgtgtgcacgaaccccccgttcagcccgaccgctgcgccttatccggtaactatcgtcttgagtccaacccggtaagacacgacttatcgccactggcagcagccactggtaacaggattagcagagcgaggtatgtaggcggtgctacagagttcttgaagtggtggcctaactacggctacactagaagaacagtatttggtatctgcgctctgctgaagccagttaccttcggaaaaagagttggtagctcttgatccggcaaacaaaccaccgctggtagcggtggtttttttgtttgcaagcagcagattacgcgcagaaaaaaaggatctcaagaagatcctttgatcttttctacggggtctgacgctcagtggaacgaaaactcacgttaagggattttggtcatgagattatcaaaaaggatcttcacctagatccttttaaattaaaaatgaagttttaaatcaatctaaagtatatatgagtaaacttggtctgacagttattagaaaaattcatccagcagacgataaaacgcaatacgctggctatccggtgccgcaatgccatacagcaccagaaaacgatccgcccattcgccgcccagttcttccgcaatatcacgggtggccagcgcaatatcctgataacgatccgccacgcccagacggccgcaatcaataaagccgctaaaacggccattttccaccataatgttcggcaggcacgcatcaccatgggtcaccaccagatcttcgccatccggcatgctcgctttcagacgcgcaaacagctctgccggtgccaggccctgatgttcttcatccagatcatcctgatccaccaggcccgcttccatacgggtacgcgcacgttcaatacgatgtttcgcctgatgatcaaacggacaggtcgccgggtccagggtatgcagacgacgcatggcatccgccataatgctcactttttctgccggcgccagatggctagacagcagatcctgacccggcacttcgcccagcagcagccaatcacggcccgcttcggtcaccacatccagcaccgccgcacacggaacaccggtggtggccagccagctcagacgcgccgcttcatcctgcagctcgttcagcgcaccgctcagatcggttttcacaaacagcaccggacgaccctgcgcgctcagacgaaacaccgccgcatcagagcagccaatggtctgctgcgcccaatcatagccaaacagacgttccacccacgctgccgggctacccgcatgcaggccatcctgttcaatcatactcttcctttttcaatattattgaagcatttatcagggttattgtctcatgagcggatacatatttgaatgtatttagaaaaataaacaaataggggttccgcgcacatttccccgaaaagtgccac

SEQ ID NO: 11 - DNA, 17 bp, Artificial Sequence
  DNA sequence of T7 Promoter
taatacgactcactata

SEQ ID NO: 12 - DNA, 20 bp, Artificial Sequence
  DNA sequence of Forward Primer for IVT template generation
gctgcaaggcgattaagttg

SEQ ID NO: 13 - DNA, 143 bp, Artificial Sequence
  DNA sequence of Reverse Primer for IVT template generation
  misc_feature (1)..(3): T is 2'-O-Methyluridine
ttttttttttttttttttttttttttttttttttttttttttttttttttttttttttttttttttttttttttttttttttttttttttttttttttttttttttttttttttttttttcagctatgaccatgttaatgcag

SEQ ID NO: 14 - DNA, 21 bp, Artificial Sequence
  DNA sequence of Forward qPCR Primer
cggtctgaggagcccttctag

SEQ ID NO: 15 - DNA, 25 bp, Artificial Sequence
  DNA sequence of Reverse qPCR Primer
cgacagaggcttctacttcaacaag

SEQ ID NO: 16 - DNA, 16 bp, Artificial Sequence
  DNA sequence of qPCR Probe
  misc_feature (1)..(1): Fluoescent label at 5'
  misc_feature (16)..(16): MGB-Q500 (Quencher) at 3'
ctgctgccgtagcctg